European Patent Specification EP 4 081 653 B1, published July 3, 2024. Title: METHODS FOR LONG READ SEQUENCING. Applicant: Singular Genomics Systems, Inc. The sequence listing filed with the application follows.

SEQUENCE LISTING (10 sequences)

SEQ ID NO: 1 - DNA, 116 bp, Artificial Sequence
  Synthetic construct
gcttccttgctggtcagattggtcgtcttattaccatttcaactactccggttatcgctggcgactccttcgagatggacgccgttggcgctctccgtctttctccattgcgtcgt

SEQ ID NO: 2 - DNA, 193 bp, Artificial Sequence
  Synthetic construct
attgttcgcgtttaccttgcgtgtacgcgcaggaaacactgacgttcttactgacgcagaagaaaacgtgcgtcaaaaattacgtgcggaaggagtgatgtaatgtctaaaggtaaaaaacgttctggcgctcgccctggtcgtccgcagccgttgcgaggtactaaaggcaagcgtaaaggcgctcgtcttt

SEQ ID NO: 3 - DNA, 297 bp, Artificial Sequence
  Synthetic construct
tgacattttaaaagagcgtggattactatctgagtccgatgctgttcaaccactaataggtaagaaatcatgagtcaagttactgaacaatccgtacgtttccagaccgctttggcctctattaagctcattcaggcttctgccgttttggatttaaccgaagatgatttcgattttctgacgagtaacaaagtttggattgctactgaccgctctcgtgctcgtcgctgcgttgaggcttgcgtttatggtacgctggactttgtgggataccctcgctttcctgctcctgttgag

SEQ ID NO: 4 - DNA, 394 bp, Artificial Sequence
  Synthetic construct
tcaagatgatgctcgttatggtttccgttgctgccatctcaaaaacatttggactgctccgcttcctcctgagactgagctttctcgccaaatgacgacttctaccacatctattgacattatgggtctgcaagctgcttatgctaatttgcatactgaccaagaacgtgattacttcatgcagcgttaccatgatgttatttcttcatttggaggtaaaacctcttatgacgctgacaaccgtcctttacttgtcatgcgctctaatctctgggcatctggctatgatgttgatggaactgaccaaacgtcgttaggccagttttctggtcgtgttcaacagacctataaacattctgtgccgcgtttctttgttcctgagcatggcactatg

SEQ ID NO: 5 - DNA, 277 bp, Artificial Sequence
  Synthetic construct
cgttcgtcaaggactggtttagatatgagtcacattttgttcatggtagagattctcttgttgacattttaaaagagcgtggattactatctgagtccgatgctgttcaaccactaataggtaagaaatcatgagtcaagttactgaacaatccgtacgtttccagaccgctttggcctctattaagctcattcaggcttctgccgttttggatttaaccgaagatgatttcgattttctgacgagtaacaaagtttggattgctactgaccgctct

SEQ ID NO: 6 - DNA, 259 bp, Artificial Sequence
  Synthetic construct
cctttcgccatcaactaacgattctgtcaaaaactgacgcgttggatgaggagaagtggcttaatatgcttggcacgttcgtcaaggactggtttagatatgagtcacattttgttcatggtagagattctcttgttgacattttaaaagagcgtggattactatctgagtccgatgctgttcaaccactaataggtaagaaatcatgagtcaagttactgaacaatccgtacgtttccagaccgctttggcctctatt

SEQ ID NO: 7 - DNA, 291 bp, Artificial Sequence
  Synthetic construct
ctgccgttttggatttaaccgaagatgatttcgattttctgacgagtaacaaagtttggattgctactgaccgctctcgtgctcgtcgctgcgttgaggcttgcgtttatggtacgctggactttgtgggataccctcgctttcctgctcctgttgagtttattgctgccgtcattgcttattatgttcatcccgtcaacattcaaacggcctgtctcatcatggaaggcgctgaatttacggaaaacattattaatggcgtcgagcgtccggttaaagccgctgaattgt

SEQ ID NO: 8 - DNA, 398 bp, Artificial Sequence
  Synthetic construct
acattcaaacggcctgtctcatcatggaaggcgctgaatttacggaaaacattattaatggcgtcgagcgtccggttaaagccgctgaattgttcgcgtttaccttgcgtgtacgcgcaggaaacactgacgttcttactgacgcagaagaaaacgtgcgtcaaaaattacgtgcggaaggagtgatgtaatgtctaaaggtaaaaaacgttctggcgctcgccctggtcgtccgcagccgttgcgaggtactaaaggcaagcgtaaaggcgctcgtctttggtatgtaggtggtcaacaattttaattgcaggggcttcggccccttacttgaggataaattatgtctaatattcaaactggcgccgagcgtatgccgcatgacctttcccatcttg

SEQ ID NO: 9 - DNA, 68 bp, Artificial Sequence
  Synthetic construct
cgtgaccctcaggtgatgcgccagggccggctgccgtcggggacagggctttccatagccatggccca

SEQ ID NO: 10 - DNA, 10 bp, Artificial Sequence
  Synthetic construct
tatatatata